European Patent Application EP 4 112 636 A1, published January 4, 2023. Title: TUMOR IMMUNE ENHANCER, AND PREPARATION METHOD THEREFOR AND APPLICATION THEREOF. Applicant: WUXI PLB THERAPEUTICS TECHNOLOGY LIMITED. CO. The sequence listing filed with the application follows.

SEQUENCE LISTING (13 sequences)

SEQ ID NO: 1 - protein, 24 aa, Artificial Sequence
  tumor immune enhancing polypeptide
LSELKTVTGTNPVFAGANYAAWAV

SEQ ID NO: 2 - protein, 24 aa, Artificial Sequence
  tumor immune enhancing polypeptide
TGTNPVFAGANYAAWAVNVAQVID

SEQ ID NO: 3 - protein, 27 aa, Artificial Sequence
  tumor immune enhancing polypeptide
SIALSSLMVAQAIPLVGELVDIGFAAY

SEQ ID NO: 4 - protein, 23 aa, Artificial Sequence
  tumor immune enhancing polypeptide
ITAENTPLPIAGVLLPTIPGKLD

SEQ ID NO: 5 - protein, 22 aa, Artificial Sequence
  tumor immune enhancing polypeptide
TTAALSILPGIGSVMGIADGAV

SEQ ID NO: 6 - protein, 24 aa, Artificial Sequence
  tumor immune enhancing polypeptide
IVAQSIALSSLMVAQAIPLVGELV

SEQ ID NO: 7 - protein, 24 aa, Artificial Sequence
  tumor immune enhancing polypeptide
GELVDIGFAAYNFVESIINLFQVV

SEQ ID NO: 8 - protein, 16 aa, Artificial Sequence
  tumor immune enhancing polypeptide
TNSVDDALINSTKIYS

SEQ ID NO: 9 - protein, 16 aa, Artificial Sequence
  tumor immune enhancing polypeptide
KAIHLVNNESSEVIVH

SEQ ID NO: 10 - protein, 27 aa, Artificial Sequence
  neoantigen peptide
WLPQAKVPFSEETQNLILPYISDMNFV

SEQ ID NO: 11 - protein, 27 aa, Artificial Sequence
  neoantigen peptide
LVLSFVGQTRVLMINGEEVEETELMGF

SEQ ID NO: 12 - protein, 27 aa, Artificial Sequence
  neoantigen peptide
RGQSQLFSLNPRGRSLVTAGRIDREEL

SEQ ID NO: 13 - protein, 27 aa, Artificial Sequence
  neoantigen peptide
SSPDEVALVEGVQSLGFTYLRLKDNYM